European Patent Specification EP 4 599 248 B1, published January 28, 2026. Title: LECTIN-BASED ASSAY FOR DETECTING MICROBIAL CONTAMINATION. Applicant: The Antibody Lab GmbH. Application EP, filed December 19, 2023. The sequence listing filed with the application follows.

SEQUENCE LISTING (16 sequences)

SEQ ID NO: 1 - protein, 228 aa, Homo sapiens
ETVTCEDAQKTCPAVIACSSPGINGFPGKDGRDDTKGEKGEPGQGLRGLQGPPGKLGPPGNPGPSGSPGPKGQKGDPGKSPDGDSSLAASERKALQTEMARIKKWLTFSLGKQVGNKFFLTNGEIMTFEKVKALCVKFQASVATPRNAAENGAIQNLIKEEAFLGITDEKTEGQFVDLTGNRLTYTNWNEGEPNNAGSDEDCVLLLKNGQWNDVPCSTSHLAVCEFPI

SEQ ID NO: 2 - protein, 222 aa, Mus musculus
SSGSQTCEDTLKTCSVIACGRDGRDGPKGEKGEPGQGLRGLQGPPGKLGPPGSVGSPGSPGPKGQKGDHGDNRAIEEKLANMEAEIRILKSKLQLTNKLHAFSMGKKSGKKLFVTNHEKMPFSKVKSLCTELQGTVAIPRNAEENKAIQEVATGIAFLGITDEATEGQFMYVTGGRLTYSNWKKDEPNNHGSGEDCVIILDNGLWNDISCQASFKAVCEFPA

SEQ ID NO: 3 - protein, 226 aa, Mus musculus
ETLTEGVQNSCPVVTCSSPGLNGFPGKDGRDGAKGEKGEPGQGLRGLQGPPGKVGPTGPPGNPGLKGAVGPKGDRGDRAEFDTSEIDSEIAALRSELRALRNWVLFSLSEKVGKKYFVSSVKKMSLDRVKALCSEFQGSVATPRNAEENSAIQKVAKDIAYLGITDVRVEGSFEDLTGNRVRYTNWNDGEPNNTGDGEDCVVILGNGKWNDVPCSDSFLAICEFSD

SEQ ID NO: 4 - protein, 229 aa, Bovine
DTETENCENIRKTCPVIACGPPGINGIPGKDGRDGAKGEKGEPGQGLRGSQGPPGKMGPQGTPGIPGIPGPIGQKGDPGENMGDYIRLATSERATLQSELNQIKNWLIFSLGKRVGKKAFFTNGKKMPFNEVKTLCAQFQGRVATPMNAEENRALKDLVTEEAFLGITDQETEGKFVDLTGKGVTYQNWNDGEPNNASPGEHCVTLLSDGTWNDIACSASFLTVCEFSL

SEQ ID NO: 5 - protein, 346 aa, Homo sapiens
QVSKVPSSISQEQSRQDAIYQNLTQLKAAVGELSEKSKLQEIYQELTQLKAAVGELPEKSKLQEIYQELTRLKAAVGELPEKSKLQEIYQELTWLKAAVGELPEKSKMQEIYQELTRLKAAVGELPEKSKQQEIYQELTRLKAAVGELPEKSKQQEIYQELTRLKAAVGELPEKSKQQEIYQELTQLKAAVERLCHPCPWEWTFFQGNCYFMSNSQRNWHDSITACKEVGAQLVVIKSAEEQNFLQLQSSRSNRFTWMGLSDLNQEGTWQWVDGSPLLPSFKQYWNRGEPNNVGEEDCAEFSGNGWNDDKCNLAKFWICKKSAASCSRDEEQFLSPAPATPNPPPA

SEQ ID NO: 6 - protein, 156 aa, Homo sapiens
GDPGKSPDGDSSLAASERKALQTEMARIKKWLTFSLGKQVGNKFFLTNGEIMTFEKVKALCVKFQASVATPRNAAENGAIQNLIKEEAFLGITDEKTEGQFVDLTGNRLTYTNWNEGEPNNAGSDEDCVLLLKNGQWNDVPCSTSHLAVCEFPILE

SEQ ID NO: 7 - protein, 162 aa, synthetic construct
GDPGKSPDGDSSLAASERKALQTEMARIKKWLTFSLGKQVGNKFFLTNGEIMTFEKVKALCVKFQASVATPRNAAENGAIQNLIKEEAFLGITDEKTEGQFVDLTGNRLTYTNWNEGEPNNAGSDEDCVLLLKNGQWNDVPCSTSHLAVCEFPILEHHHHHH

SEQ ID NO: 8 - protein, 240 aa, synthetic construct
MHHHHHHHHHHDTETENCENIRKTCPVIACGPPGINGIPGKDGRDGAKGEKGEPGQGLRGSQGPPGKMGPQGTPGIPGIPGPIGQKGDPGENMGDYIRLATSERATLQSELNQIKNWLIFSLGKRVGKKAFFTNGKKMPFNEVKTLCAQFQGRVATPMNAEENRALKDLVTEEAFLGITDQETEGKFVDLTGKGVTYQNWNDGEPNNASPGEHCVTLLSDGTWNDIACSASFLTVCEFSL

SEQ ID NO: 9 - protein, 236 aa, synthetic construct
ETVTCEDAQKTCPAVIACSSPGINGFPGKDGRDGTKGEKGEPGQGLRGLQGPPGKLGPPGNPGPSGSPGPKGQKGDPGKSPDGDSSLAASERKALQTEMARIKKWLTFSLGKQVGNKFFLTNGEIMTFEKVKALCVKFQASVATPRNAAENGAIQNLIKEEAFLGITDEKTEGQFVDLTGNRLTYTNWNEGEPNNAGSDEDCVLLLKNGQWNDVPCSTSHLAVCEFPILEHHHHHH

SEQ ID NO: 10 - protein, 112 aa, Homo sapiens
VGNKFFLTNGEIMTFEKVKALCVKFQASVATPRNAAENGAIQNLIKEEAFLGITDEKTEGQFVDLTGNRLTYTNWNEGEPNNAGSDEDCVLLLKNGQWNDVPCSTSHLAVCE

SEQ ID NO: 11 - protein, 96 aa, Mus musculus
SLCTELQGTVAIPRNAEENKAIQEVATGIAFLGITDEATEGQFMYVTGGRLTYSNWKKDEPNNHGSGEDCVIILDNGLWNDISCQASFKAVCEFPA

SEQ ID NO: 12 - protein, 113 aa, Mus musculus
KVGKKYFVSSVKKMSLDRVKALCSEFQGSVATPRNAEENSAIQKVAKDIAYLGITDVRVEGSFEDLTGNRVRYTNWNDGEPNNTGDGEDCVVILGNGKWNDVPCSDSFLAICE

SEQ ID NO: 13 - protein, 112 aa, Bovine
VGKKAFFTNGKKMPFNEVKTLCAQFQGRVATPMNAEENRALKDLVTEEAFLGITDQETEGKFVDLTGKGVTYQNWNDGEPNNASPGEHCVTLLSDGTWNDIACSASFLTVCE

SEQ ID NO: 14 - protein, 116 aa, Homo sapiens
FQGNCYFMSNSQRNWHDSITACKEVGAQLVVIKSAEEQNFLQLQSSRSNRFTWMGLSDLNQEGTWQWVDGSPLLPSFKQYWNRGEPNNVGEEDCAEFSGNGWNDDKCNLAKFWICK

SEQ ID NO: 15 - skipped

SEQ ID NO: 16 - protein, 273 aa, synthetic construct
MKWVTFISLLFLFSSAYSSLFPSLPLLLLSMVAASYSETVTCEDAQKTCPAVIACSSPGINGFPGKDGRDGTKGEKGEPGQGLRGLQGPPGKLGPPGNPGPSGSPGPKGQKGDPGKSPDGDSSLAASERKALQTEMARIKKWLTFSLGKQVGNKFFLTNGEIMTFEKVKALCVKFQASVATPRNAAENGAIQNLIKEEAFLGITDEKTEGQFVDLTGNRLTYTNWNEGEPNNAGSDEDCVLLLKNGQWNDVPCSTSHLAVCEFPILEHHHHHH